European Patent Specification EP 4 056 692 B1, published October 29, 2025. Title: Novel 5,10-methylenetetrahydrofolate reductase variant and a method for producing L-valine using the same. Applicant: CJ CheilJedang Corporation. The sequence listing filed with the application follows.

SEQUENCE LISTING (11 sequences)

SEQ ID NO: 1 - protein, 294 aa, Artificial Sequence
  5,10-methylenetetrahydrofolate reductase variant
MPPHDDAAEERLYRAAEVFHDLGASFVSVTYGAGGSTRERTSRIARRLAKQPLTTLVHLTLVNHTREEMKAILREYLELGLTNLLALRGDPPGDPLGDWVSTDGGLNYASELIDLIKSTPEFREFDLGIASFPEGHFRAKTLEEDTKYTLAKLRGGAEYSITQMFFDVEDYLRLRDRLVAADPIHGAKPIIPGIMPITSLRSVRRQVELSGAQLPSQLEESLVRAANGNEEANKDEIRKVGIEYSTNMAERLIAEGAEDLHFMTLNFTRATQEVLYNLGMAPAWGAEHGQDAVR

SEQ ID NO: 2 - DNA, 885 bp, Artificial Sequence
  5,10-methylenetetrahydrofolate reductase variant coding gene
atgccaccccacgatgatgcagctgaagagcgtctttaccgagcagcagaggtcttccatgacctcggtgcatcgtttgtctccgtgacttatggtgctggcggatcaacccgtgagagaacctcacgtattgctcgacgattagcgaaacaaccgttgaccactctggtgcacctgaccctggttaaccacactcgcgaagagatgaaggcaattcttcgggaatacctagagctgggattaacaaacctgttggcgcttcgaggagatccgcctggagacccattaggcgattgggtgagcaccgatggaggactgaactacgcctctgagctcatcgatcttattaagtccactcctgagttccgggaattcgacctcggtatcgcctccttccccgaagggcatttccgggcgaaaactctagaagaagacaccaaatacactctggcgaagctgcgtggaggtgcagagtactccatcacgcagatgttctttgatgtggaagactacctgcgacttcgtgatcgccttgtcgctgcagaccccattcatggcgcgaagccaatcattcctggcatcatgcccattacgagcctgcggtctgtgcgtcgacaggtcgaactctctggtgctcaattgccgagccaactagaagaatcacttgttcgagctgcaaacggcaatgaagaagcgaacaaagacgagatccgcaaggtgggcattgaatattccaccaatatggcagagcgactcattgccgaaggtgcggaagatctgcacttcatgacgcttaacttcacccgtgcaacccaagaagtgttgtacaaccttggcatggcgcctgcttggggagcagagcacggccaagacgcggtgcgttaa

SEQ ID NO: 3 - protein, 294 aa, Artificial Sequence
  Wild-type 5,10-methylenetetrahydrofolate reductase
MPPRDDAAEERLYRAAEVFHDLGASFVSVTYGAGGSTRERTSRIARRLAKQPLTTLVHLTLVNHTREEMKAILREYLELGLTNLLALRGDPPGDPLGDWVSTDGGLNYASELIDLIKSTPEFREFDLGIASFPEGHFRAKTLEEDTKYTLAKLRGGAEYSITQMFFDVEDYLRLRDRLVAADPIHGAKPIIPGIMPITSLRSVRRQVELSGAQLPSQLEESLVRAANGNEEANKDEIRKVGIEYSTNMAERLIAEGAEDLHFMTLNFTRATQEVLYNLGMAPAWGAEHGQDAVR

SEQ ID NO: 4 - DNA, 885 bp, Artificial Sequence
  Wild-type 5,10-methylenetetrahydrofolate reductase coding gene
atgccaccccgcgatgatgcagctgaagagcgtctttaccgagcagcagaggtcttccatgacctcggtgcatcgtttgtctccgtgacttatggtgctggcggatcaacccgtgagagaacctcacgtattgctcgacgattagcgaaacaaccgttgaccactctggtgcacctgaccctggttaaccacactcgcgaagagatgaaggcaattcttcgggaatacctagagctgggattaacaaacctgttggcgcttcgaggagatccgcctggagacccattaggcgattgggtgagcaccgatggaggactgaactacgcctctgagctcatcgatcttattaagtccactcctgagttccgggaattcgacctcggtatcgcctccttccccgaagggcatttccgggcgaaaactctagaagaagacaccaaatacactctggcgaagctgcgtggaggtgcagagtactccatcacgcagatgttctttgatgtggaagactacctgcgacttcgtgatcgccttgtcgctgcagaccccattcatggcgcgaagccaatcattcctggcatcatgcccattacgagcctgcggtctgtgcgtcgacaggtcgaactctctggtgctcaattgccgagccaactagaagaatcacttgttcgagctgcaaacggcaatgaagaagcgaacaaagacgagatccgcaaggtgggcattgaatattccaccaatatggcagagcgactcattgccgaaggtgcggaagatctgcacttcatgacgcttaacttcacccgtgcaacccaagaagtgttgtacaaccttggcatggcgcctgcttggggagcagagcacggccaagacgcggtgcgttaa

SEQ ID NO: 5 - DNA, 36 bp, Artificial Sequence
  metF_1F
tcgagctcggtacccttcagaagaattcttatggcc

SEQ ID NO: 6 - DNA, 44 bp, Artificial Sequence
  metF_2R
ctcttcagctgcatcatcgtggggtggcataaactcgacagaaa

SEQ ID NO: 7 - DNA, 44 bp, Artificial Sequence
  metF_3F
tttctgtcgagtttatgccaccccacgatgatgcagctgaagag

SEQ ID NO: 8 - DNA, 36 bp, Artificial Sequence
  metF_4R
ctctagaggatccccatcaaagaacatctgcgtgat

SEQ ID NO: 9 - DNA, 21 bp, Artificial Sequence
  metF_5F
ttcagaagaattcttatggcc

SEQ ID NO: 10 - DNA, 21 bp, Artificial Sequence
  metF_6R
atcaaagaacatctgcgtgat

SEQ ID NO: 11 - DNA, 5803 bp, Artificial Sequence
  pDCM2
gttcgcttgctgtccataaaaccgcccagtctagctatcgccatgtaagcccactgcaagctacctgctttctctttgcgcttgcgttttcccttgtccagatagcccagtagctgacattcatccggggtcagcaccgtttctgcggactggctttctacgtgttccgcttcctttagcagcccttgcgccctgagtgcttgcggcagcgtgaagctagcttttatcgccattcgccattcaggctgcgcaactgttgggaagggcgatcggtgcgggcctcttcgctattacgccagctggcgaaagggggatgtgctgcaaggcgattaagttgggtaacgccagggttttcccagtcacgacgttgtaaaacgacggccagtgaattcgagctcggtacccggggatcctctagagtcgacctgcaggcatgcaagcttggcgtaatcatggtcatagctgtttcctgtgtgaaattgttatccgctcacaattccacacaacatacgagccggaagcataaagtgtaaagcctggggtgcctaatgagtgagctaactcacattaattgcgttgcgctcactgcccgctttccagtcgggaaacctgtcgtgccagctgcattaatgaatcggccaacgcgcggggagaggcggtttgcgtattgggcgctcttccgcttcctcgctcactgactcgctgcgctcggtcgttcggctgcggcgagcggtatcagctcactcaaaggcggtaatacggttatccacagaatcaggggataacgcaggaaagaacatgtgagcaaaaggccagcaaaaggccaggaaccgtaaaaaggccgcgttgctggcgtttttccataggctccgcccccctgacgagcatcacaaaaatcgacgctcaagtcagaggtggcgaaacccgacaggactataaagataccaggcgtttccccctggaagctccctcgtgcgctctcctgttccgaccctgccgcttaccggatacctgtccgcctttctcccttcgggaagcgtggcgctttctcaatgctcacgctgtaggtatctcagttcggtgtaggtcgttcgctccaagctgggctgtgtgcacgaaccccccgttcagcccgaccgctgcgccttatccggtaactatcgtcttgagtccaacccggtaagacacgacttatcgccactggcagcagccactggtaacaggattagcagagcgaggtatgtaggcggtgctacagagttcttgaagtggtggcctaactacggctacactagaaggacagtatttggtatctgcgctctgctgaagccagttaccttcggaaaaagagttggtagctcttgatccggcaaacaaaccaccgctggtagcggtggtttttttgtttgcaagcagcagattacgcgcagaaaaaaaggatctcaagaagatcctttgatcttttctacggggtctgacgctcagtggaacgaaaactcacgttaagggattttggtcatgagattatcaaaaaggatcttcacctagatccttttggggtgggcgaagaactccagcatgagatccccgcgctggaggatcatccagccctgatagaaacagaagccactggagcacctcaaaaacaccatcatacactaaatcagtaagttggcagcatcacccgacgcactttgcgccgaataaatacctgtgacggaagatcacttcgcagaataaataaatcctggtgtccctgttgataccgggaagccctgggccaacttttggcgaaaatgagacgttgatcggcacgtaagaggttccaactttcaccataatgaaataagatcactaccgggcgtattttttgagttatcgagattttcaggagctgatagaaacagaagccactggagcacctcaaaaacaccatcatacactaaatcagtaagttggcagcatcacccgacgcactttgcgccgaataaatacctgtgacggaagatcacttcgcagaataaataaatcctggtgtccctgttgataccgggaagccctgggccaacttttggcgaaaatgagacgttgatcggcacgtaagaggttccaactttcaccataatgaaataagatcactaccgggcgtattttttgagttatcgagattttcaggagctctttggcatcgtctctcgcctgtcccctcagttcagtaatttcctgcatttgcctgtttccagtcggtagatattccacaaaacagcagggaagcagcgcttttccgctgcataaccctgcttcggggtcattatagcgattttttcggtatatccatcctttttcgcacgatatacaggattttgccaaagggttcgtgtagactttccttggtgtatccaacggcgtcagccgggcaggataggtgaagtaggcccacccgcgagcgggtgttccttcttcactgtcccttattcgcacctggcggtgctcaacgggaatcctgctctgcgaggctggccggctaccgccggcgtaacagatgagggcaagcggatggctgatgaaaccaagccaaccaggaagggcagcccacctatcaaggtgtactgccttccagacgaacgaagagcgattgaggaaaaggcggcggcggccggcatgagcctgtcggcctacctgctggccgtcggccagggctacaaaatcacgggcgtcgtggactatgagcacgtccgcgagggcgtcccggaaaacgattccgaagcccaacctttcatagaaggcggcggtggaatcgaaatctcgtgatggcaggttgggcgtcgcttggtcggtcatttcgaaaaaggttaggaatacggttagccatttgcctgcttttatatagttcantatgggattcacctttatgttgataagaaataaaagaaaatgccaataggatatcggcattttcttttgcgtttttatttgttaactgttaattgtccttgttcaaggatgctgtctttgacaacagatgttttcttgcctttgatgttcagcaggaagctcggcgcaaacgttgattgtttgtctgcgtagaatcctctgtttgtcatatagcttgtaatcacgacattgtttcctttcgcttgaggtacagcgaagtgtgagtaagtaaaggttacatcgttaggcggatcaagatccatttttaacacaaggccagttttgttcagcggcttgtatgggccagttaaagaattagaaacataaccaagcatgtaaatatcgttagacgtaatgccgtcaatcgtcatttttgatccgcgggagtcagtgaacaggtaccatttgccgttcattttaaagacgttcgcgcgttcaatttcatctgttactgtgttagatgcaatcagcggtttcatcacttttttcagtgtgtaatcatcgtttagctcaatcataccgagagcgccgtttgctaactcagccgtgcgttttttatcgctttgcagaagtttttgactttcttgacggaagaatgatgtgcttttgccatagtatgctttgttaaataaagattcttcgccttggtagccatcttcagttccagtgtttgcttcaaatactaagtatttgtggcctttatcttctacgtagtgaggatctctcagcgtatggttgtcgcctgagctgtagttgccttcatcgatgaactgctgtacattttgatacgtttttccgtcaccgtcaaagattgatttataatcctctacaccgttgatgttcaaagagctgtctgatgctgatacgttaacttgtgcagttgtcagtgtttgtttgccgtaatgtttaccggagaaatcagtgtagaataaacggatttttccgtcagatgtaaatgtggctgaacctgaccattcttgtgtttggtcttttaggatagaatcatttgcatcgaatttgtcgctgtctttaaagacgcggccagcgtttttccagctgtcaatagaagtttcgccgactttttgatagaacatgtaaatcgatgtgtcatccgcatttttaggatctccggctaatgcaaagacgatgtggtagccgtgatagtttgcgacagtgccgtcagcgttttgtaatggccagctgtcccaaacgtccaggccttttgcagaagagatatttttaattgtggacgaatcaaattcagaaacttgatatttttcatttttttgctgttcagggatttgcagcatatcatggcgtgtaatatgggaaatgccgtatgtttccttatatggcttttggttcgtttctttcgcaaacgcttgagttgcgcctcctgccagcagtgcggtagtaaaggttaatactgttgcttgttttgcaaactttttgatgttcatcgttcatgtctccttttttatgtactgtgttagcggtctgcttcttccagccctcctgtttgaagatggcaagttagttacgcacaataaaaaaagacctaaaatatgtaaggggtgacgccaaagtatacactttgccctttacacattttaggtcttgcctgctttatcagtaacaaacccgcgcgatttacttttcgacctcattctattagactctcgtttggattgcaactggtctattttcctcttttgtttgatagaaaatcataaaaggatttgcagactacgggcctaaagaactaaaaaatctatctgtttcttttcattctctgtattttttatagtttctgttgcatgggcataaagttgcctttttaatcacaattcagaaaatatcataatatctcatttcactaaataatagtgaacggcaggtatatgtgatgggttaaaaaggatcaccccagagtcccgctcagaagaactcgtcaagaaggcgatagaaggcgatgcgctgcgaatcgggagcggcgataccgtaaagcacgaggaagcggtcagcccattcgccgccaagctcttcagcaatatcacgggtagccaacgctatgtcctgatagcggtccgccacacccagccggccacagtcgatgaatccagaaaagcggccattttccaccatgatattcggcaagcaggcatcgccatgggtcacgacgagatcctcgccgtcgggcatccgcgccttgagcctggcgaacagttcggctggcgcgagcccctgatgctcttcgtccagatcatcctgatcgacaagaccggcttccatccgagtacgtgctcgctcgatgcgatgtttcgcttggtggtcgaatgggcaggtagccggatcaagcgtatgcagccgccgcattgcatcagccatgatggatactttctcggcaggagcaaggtgagatgacaggagatcctgccccggcacttcgcccaatagcagccagtcccttcccgcttcagtgacaacgtcgagacagctgcgcaaggaacgcccgtcgtggccagccacgatagccgcgctgcctcgtcttggagttcattcagggcaccggacaggtcggtcttgacaaaaagaaccgggcgcccctgcgctgacagccggaacacggcggcatcagagcagccgattgtctgttgtgcccagtcatagccgaatagcctctccacccaagcggccggagaacctgcgtgcaatccatcttgttcaatcatgcgaaacgatcctcatcctgtctcttgatcagatcttgatcccctgcgccatcagatccttggcggcaagaaagccatccagtttactttgcagggcttcccaaccttaccagagggcgccccagctggcaattccg